European Patent Specification EP 3 794 041 B1, published July 12, 2023. Title: Anti-MUC1 antibody. Applicant: Glycotope GmbH. The sequence listing filed with the application follows.

SEQUENCE LISTING (23 sequences)

SEQ ID NO: 1 - protein, 5 aa, Artificial Sequence
  CDR-H1
NYWMN

SEQ ID NO: 2 - protein, 19 aa, Artificial Sequence
  CDR-H2
  VARIANT (8)..(8): Xaa is any amino acid except Asn
EIRLKSNXYTTHYAESVKG

SEQ ID NO: 3 - protein, 6 aa, Artificial Sequence
  CDR-H3
HYYFDY

SEQ ID NO: 4 - protein, 16 aa, Artificial Sequence
  CDR-L1
RSSKSLLHSNGITYFF

SEQ ID NO: 5 - protein, 7 aa, Artificial Sequence
  CDR-L2
QMSNLAS

SEQ ID NO: 6 - protein, 9 aa, Artificial Sequence
  CDR-L3
AQNLELPPT

SEQ ID NO: 7 - protein, 19 aa, Artificial Sequence
  CDR-H2
EIRLKSNQYTTHYAESVKG

SEQ ID NO: 8 - protein, 19 aa, Artificial Sequence
  CDR-H2
EIRLKSNNYTTHYAESVKG

SEQ ID NO: 9 - protein, 117 aa, Artificial Sequence
  heavy chain variable region
  VARIANT (57)..(57): Xaa is any amino acid except Asn
EVQLVESGGGLVQPGGSMRLSCVASGFPFSNYWMNWVRQAPGKGLEWVGEIRLKSNXYTTHYAESVKGRFTISRDDSKNSLYLQMNSLKTEDTAVYYCTRHYYFDYWGQGTLVTVSS

SEQ ID NO: 10 - protein, 117 aa, Artificial Sequence
  heavy chain variable region
EVQLVESGGGLVQPGGSMRLSCVASGFPFSNYWMNWVRQAPGKGLEWVGEIRLKSNQYTTHYAESVKGRFTISRDDSKNSLYLQMNSLKTEDTAVYYCTRHYYFDYWGQGTLVTVSS

SEQ ID NO: 11 - protein, 117 aa, Artificial Sequence
  heavy chain variable region
EVQLVESGGGLVQPGGSMRLSCVASGFPFSNYWMNWVRQAPGKGLEWVGEIRLKSNNYTTHYAESVKGRFTISRDDSKNSLYLQMNSLKTEDTAVYYCTRHYYFDYWGQGTLVTVSS

SEQ ID NO: 12 - protein, 113 aa, Artificial Sequence
  light chain variable region
DIVMTQSPLSNPVTPGEPASISCRSSKSLLHSNGITYFFWYLQKPGQSPQLLIYQMSNLASGVPDRFSGSGSGTDFTLRISRVEAEDVGVYYCAQNLELPPTFGQGTKVEIKR

SEQ ID NO: 13 - protein, 4 aa, Artificial Sequence
  epitope
PDTR

SEQ ID NO: 14 - protein, 4 aa, Artificial Sequence
  epitope
PESR

SEQ ID NO: 15 - protein, 447 aa, Artificial Sequence
  heavy chain
  VARIANT (57)..(57): Xaa is any amino acid except Asn
EVQLVESGGGLVQPGGSMRLSCVASGFPFSNYWMNWVRQAPGKGLEWVGEIRLKSNXYTTHYAESVKGRFTISRDDSKNSLYLQMNSLKTEDTAVYYCTRHYYFDYWGQGTLVTVSSASTKGPSVFPLAPSSKSTSGGTAALGCLVKDYFPEPVTVSWNSGALTSGVHTFPAVLQSSGLYSLSSVVTVPSSSLGTQTYICNVNHKPSNTKVDKKVEPKSCDKTHTCPPCPAPELLGGPSVFLFPPKPKDTLMISRTPEVTCVVVDVSHEDPEVKFNWYVDGVEVHNAKTKPREEQYNSTYRVVSVLTVLHQDWLNGKEYKCKVSNKALPAPIEKTISKAKGQPREPQVYTLPPSRDELTKNQVSLTCLVKGFYPSDIAVEWESNGQPENNYKTTPPVLDSDGSFFLYSKLTVDKSRWQQGNVFSCSVMHEGLHNHYTQKSLSLSPGK

SEQ ID NO: 16 - protein, 219 aa, Artificial Sequence
  light chain
DIVMTQSPLSNPVTPGEPASISCRSSKSLLHSNGITYFFWYLQKPGQSPQLLIYQMSNLASGVPDRFSGSGSGTDFTLRISRVEAEDVGVYYCAQNLELPPTFGQGTKVEIKRTVAAPSVFIFPPSDEQLKSGTASVVCLLNNFYPREAKVQWKVDNALQSGNSQESVTEQDSKDSTYSLSSTLTLSKADYEKHKVYACEVTHQGLSSPVTKSFNRGEC

SEQ ID NO: 17 - DNA, 1401 bp, Artificial Sequence
  heavy chain
atgaagcacctgtggttctttctgctgctggtggccgctcctagatgggtgctgtctgaagtgcagctggtggaatctggcggaggattggttcagcctggcggctccatgagactgtcttgtgtggcctctggcttccccttctccaactactggatgaactgggtccgacaggcccctggcaaaggactggaatgggtcggagagatccggctgaagtccaaccagtacaccacacactacgccgagtccgtgaagggcagattcaccatctctcgggacgactccaagaactccctgtacctgcagatgaacagcctgaaaaccgaggacaccgccgtgtactactgcacccggcactactacttcgactactggggccagggcaccctggtcacagtttcttccgcttccaccaagggacccagcgtgttccctctggctccttccagcaagtctacctctggcggaacagctgctctgggctgcctggtcaaggactactttcctgagcctgtgaccgtgtcctggaactctggcgctctgacatctggcgtgcacacctttccagctgtgctgcagtcctccggcctgtactctctgtcctctgtcgtgaccgtgccttccagctctctgggaacccagacctacatctgcaatgtgaaccacaagccttccaacaccaaggtggacaagaaggtggaacccaagtcctgcgacaagacccacacctgtcctccatgtcctgctccagaactgctcggcggaccttccgtgttcctgtttcctccaaagcctaaggacaccctgatgatcagcagaacccctgaagtgacctgcgtggtggtggatgtgtctcacgaggaccccgaagtgaagttcaattggtacgtggacggcgtggaagtgcacaacgccaagaccaagcctagagaggaacagtacaactccacctacagagtggtgtccgtgctgaccgtgctgcaccaggattggctgaacggcaaagagtacaagtgcaaggtgtccaacaaggccctgcctgctcctatcgaaaagaccatctccaaggccaagggccagcctagggaaccccaggtttacaccttgcctccaagcagggacgagctgaccaagaaccaggtgtccctgacctgcctcgtgaagggattctacccctccgatatcgccgtggaatgggagtctaatggccagcctgagaacaactacaagacaacccctcctgtgctggactccgacggctcattcttcctgtactccaagctgacagtggacaagtccagatggcagcagggcaacgtgttctcctgctccgtgatgcatgagggcctgcacaaccactacacccagaagtccctgtctctgagccccggcaaatga

SEQ ID NO: 18 - DNA, 720 bp, Artificial Sequence
  light chain
atggttctgcagacacaggtgttcatctccctgctgctgtggatctctggcgcctacggcgacatcgtgatgacccagtctccactgagcaaccccgtgacacctggcgagcctgcctccatctcttgccggtcctctaagtctctgctgcactccaacggcatcacctactttttctggtatctgcagaagcccggccagtctcctcagctgctgatctaccagatgtccaacctggcctctggcgtgcccgatagattttccggctctggctctggcaccgacttcaccctgagaatctccagagtggaagccgaggacgtgggcgtgtactactgtgcccagaacctggaactgcctcctacctttggccagggcaccaaggtggaaatcaagcggacagtggccgctccttccgtgtttatcttcccaccttccgacgagcagctgaagtccggcacagcttctgtcgtgtgcctgctgaacaacttctaccctcgggaagccaaggtgcagtggaaggtggacaatgccctgcagtccggcaactcccaagagtctgtgaccgagcaggactccaaggacagcacctacagcctgtcctccacactgaccctgtccaaggccgactacgagaagcacaaggtgtacgcctgcgaagtgacccatcagggcctgtctagccctgtgaccaagtctttcaaccggggcgagtgctga

SEQ ID NO: 19 - protein, 447 aa, Artificial Sequence
  heavy chain
EVQLVESGGGLVQPGGSMRLSCVASGFPFSNYWMNWVRQAPGKGLEWVGEIRLKSNNYTTHYAESVKGRFTISRDDSKNSLYLQMNSLKTEDTAVYYCTRHYYFDYWGQGTLVTVSSASTKGPSVFPLAPSSKSTSGGTAALGCLVKDYFPEPVTVSWNSGALTSGVHTFPAVLQSSGLYSLSSVVTVPSSSLGTQTYICNVNHKPSNTKVDKKVEPKSCDKTHTCPPCPAPELLGGPSVFLFPPKPKDTLMISRTPEVTCVVVDVSHEDPEVKFNWYVDGVEVHNAKTKPREEQYNSTYRVVSVLTVLHQDWLNGKEYKCKVSNKALPAPIEKTISKAKGQPREPQVYTLPPSRDELTKNQVSLTCLVKGFYPSDIAVEWESNGQPENNYKTTPPVLDSDGSFFLYSKLTVDKSRWQQGNVFSCSVMHEGLHNHYTQKSLSLSPGK

SEQ ID NO: 20 - protein, 460 aa, Artificial Sequence
  heavy chain
  VARIANT (76)..(76): Xaa is any amino acid except Asn
MKHLWFFLLLVAAPRWVLSEVQLVESGGGLVQPGGSMRLSCVASGFPFSNYWMNWVRQAPGKGLEWVGEIRLKSNXYTTHYAESVKGRFTISRDDSKNSLYLQMNSLKTEDTAVYYCTRHYYFDYWGQGTLVTVSSAKTTPPSVYPLAPGSAAQTNSMVTLGCLVKGYFPEPVTVTWNSGSLSSGVHTFPAVLQSDLYTLSSSVTVPSSTWPSQTVTCNVAHPASSTKVDKKIVPRDCGCKPCICTVPEVSSVFIFPPKPKDVLTITLTPKVTCVVVDISKDDPEVQFSWFVDDVEVHTAQTKPREEQINSTFRSVSELPIMHQDWLNGKEFKCRVNSAAFPAPIEKTISKTKGRPKAPQVYTIPPPKEQMAKDKVSLTCMITNFFPEDITVEWQWNGQPAENYKNTQPIMDTDGSYFVYSKLNVQKSNWEAGNTFTCSVLHEGLHNHHTEKSLSHSPGK

SEQ ID NO: 21 - protein, 239 aa, Artificial Sequence
  light chain
MVLQTQVFISLLLWISGAYGDIVMTQSPLSNPVTPGEPASISCRSSKSLLHSNGITYFFWYLQKPGQSPQLLIYQMSNLASGVPDRFSGSGSGTDFTLRISRVEAEDVGVYYCAQNLELPPTFGQGTKVEIKRADAAPTVSIFPPSSEQLTSGGASVVCFLNNFYPKDINVKWKIDGSERQNGVLNSWTDQDSKDSTYSMSSTLTLTKDEYERHNSYTCEATHKTSTSPIVKSFNRNEC

SEQ ID NO: 22 - protein, 447 aa, Artificial Sequence
  heavy chain
EVQLVESGGGLVQPGGSMRLSCVASGFPFSNYWMNWVRQAPGKGLEWVGEIRLKSNQYTTHYAESVKGRFTISRDDSKNSLYLQMNSLKTEDTAVYYCTRHYYFDYWGQGTLVTVSSASTKGPSVFPLAPSSKSTSGGTAALGCLVKDYFPEPVTVSWNSGALTSGVHTFPAVLQSSGLYSLSSVVTVPSSSLGTQTYICNVNHKPSNTKVDKKVEPKSCDKTHTCPPCPAPELLGGPSVFLFPPKPKDTLMISRTPEVTCVVVDVSHEDPEVKFNWYVDGVEVHNAKTKPREEQYNSTYRVVSVLTVLHQDWLNGKEYKCKVSNKALPAPIEKTISKAKGQPREPQVYTLPPSRDELTKNQVSLTCLVKGFYPSDIAVEWESNGQPENNYKTTPPVLDSDGSFFLYSKLTVDKSRWQQGNVFSCSVMHEGLHNHYTQKSLSLSPGK

SEQ ID NO: 23 - protein, 460 aa, Artificial Sequence
  heavy chain
MKHLWFFLLLVAAPRWVLSEVQLVESGGGLVQPGGSMRLSCVASGFPFSNYWMNWVRQAPGKGLEWVGEIRLKSNQYTTHYAESVKGRFTISRDDSKNSLYLQMNSLKTEDTAVYYCTRHYYFDYWGQGTLVTVSSAKTTPPSVYPLAPGSAAQTNSMVTLGCLVKGYFPEPVTVTWNSGSLSSGVHTFPAVLQSDLYTLSSSVTVPSSTWPSQTVTCNVAHPASSTKVDKKIVPRDCGCKPCICTVPEVSSVFIFPPKPKDVLTITLTPKVTCVVVDISKDDPEVQFSWFVDDVEVHTAQTKPREEQINSTFRSVSELPIMHQDWLNGKEFKCRVNSAAFPAPIEKTISKTKGRPKAPQVYTIPPPKEQMAKDKVSLTCMITNFFPEDITVEWQWNGQPAENYKNTQPIMDTDGSYFVYSKLNVQKSNWEAGNTFTCSVLHEGLHNHHTEKSLSHSPGK